European Patent Application EP 4 202 047 A1, published June 28, 2023. Title: BCMA-BINDING SINGLE VARIABLE STRUCTURAL DOMAIN AND ANTIGEN-BINDING MOLECULE. Applicant: CHIA TAI TIANQING PHARMACEUTICAL GROUP CO., LTD. Application EP21857622.1. The sequence listing filed with the application follows.

SEQUENCE LISTING (27 sequences)

SEQ ID NO: 1 - DNA, 23 bp, Artificial Sequence
  Primer Sequence of Call001
gtcctggctgctcttctacaagg

SEQ ID NO: 2 - DNA, 23 bp, Artificial Sequence
  Primer Sequence of Call002
ggtacgtgctgttgaactgttcc

SEQ ID NO: 3 - DNA, 29 bp, Artificial Sequence
  Primer Sequence of V-Back
gatgtgcagctgcaggagtctggrggagg

SEQ ID NO: 4 - DNA, 34 bp, Artificial Sequence
  Primer Sequence of V-Fwd
ctagtgcggccgctgaggagacggtgacctgggt

SEQ ID NO: 5 - protein, 232 aa, Homo sapiens
EPKSCDKTHTCPPCPAPELLGGPSVFLFPPKPKDTLMISRTPEVTCVVVDVSHEDPEVKFNWYVDGVEVHNAKTKPREEQYNSTYRVVSVLTVLHQDWLNGKEYKCKVSNKALPAPIEKTISKAKGQPREPQVYTLPPSRDELTKNQVSLTCLVKGFYPSDIAVEWESNGQPENNYKTTPPVLDSDGSFFLYSKLTVDKSRWQQGNVFSCSVMHEALHNHYTQKSLSLSPGK

SEQ ID NO: 6 - protein, 54 aa, Homo sapiens
MLQMAGQCSQNEYFDSLLHACIPCQLRCSSNTPPLTCQRYCNASVTNSVKGTNA

SEQ ID NO: 7 - protein, 5 aa, Camelus bactrianus
PCAMG

SEQ ID NO: 8 - protein, 16 aa, Camelus bactrianus
WITVDGTTDYADSVKG

SEQ ID NO: 9 - protein, 12 aa, Camelus bactrianus
VYILTPSCRPQP

SEQ ID NO: 10 - protein, 5 aa, Camelus bactrianus
SDCMG

SEQ ID NO: 11 - protein, 17 aa, Camelus bactrianus
RIETGYGGTLYADSVKG

SEQ ID NO: 12 - protein, 17 aa, Camelus bactrianus
KRSWCSPTWWREVDYNY

SEQ ID NO: 13 - protein, 5 aa, Camelus bactrianus
MVCMG

SEQ ID NO: 14 - protein, 17 aa, Camelus bactrianus
LITTDGGTTLYADSVKG

SEQ ID NO: 15 - protein, 18 aa, Camelus bactrianus
DDRPWCMTVGVRTEDYDT

SEQ ID NO: 16 - protein, 120 aa, Camelus bactrianus
QVQLVESGGGSVQAGGSLLLSCAASGYTFSPCAMGWFRQAPGKERSLVSWITVDGTTDYADSVKGRFTISRDNAKNMVYLQMTSLEPEDTATYYCNTVYILTPSCRPQPWGPGTQVTVSS

SEQ ID NO: 17 - DNA, 360 bp, Camelus bactrianus
caggtgcagctggtggagtctgggggaggctcggtgcaggctggagggtctctattactctcctgtgcagcctctggatacaccttcagtccctgcgccatgggctggttccgccaggctccagggaaggagcgctcgttggtctcatggattactgttgatggtacaacagactatgcagactccgtgaagggccgattcaccatctcccgagacaacgccaagaacatggtgtatctgcaaatgactagtttggaacctgaggacacggccacgtattactgtaatactgtgtacattcttactccgtcctgccgcccccagccctggggcccggggacccaggtcactgtctcatca

SEQ ID NO: 18 - protein, 126 aa, Camelus bactrianus
QVQLVESGGGSVQAGGSLRLSCAASGVTFNSDCMGWFRQAPGKEREAVARIETGYGGTLYADSVKGRFTISRDNAKKTVYLQMNSLKFEDTAMYYCAAKRSWCSPTWWREVDYNYWGQGTLVTVSS

SEQ ID NO: 19 - DNA, 378 bp, Camelus bactrianus
caggtgcagctggtggagtctgggggaggctcggtgcaggctggagggtctctgagactctcctgtgcagcctctggagtcacttttaatagtgactgtatgggttggttccgccaggctccgggaaaggagcgcgaggcagtcgcacgtattgaaactggttatggtggcactctctatgccgactccgtgaagggacgattcaccatctcccgagacaacgccaagaagacggtgtatctgcaaatgaacagcctaaaatttgaggacactgccatgtactactgtgcggctaagagatcctggtgttctcctacgtggtggcgcgaagttgactataactactggggacaggggaccctggtcactgtctcatca

SEQ ID NO: 20 - protein, 127 aa, Camelus bactrianus
QVQLVESGGGSVPAGGSMRLSCAASGYRNPMVCMGWFRQAPGKKREGVALITTDGGTTLYADSVKGRFTISQDNAKNTVYLQMNNLKPEDTAMYTCAADDRPWCMTVGVRTEDYDTWGQGTLVTVSS

SEQ ID NO: 21 - DNA, 381 bp, Camelus bactrianus
caggtgcagctggtggagtctgggggaggctcggtgcctgctggagggtctatgagactctcctgtgcagcctctggttacaggaatcctatggtgtgtatgggctggtttcgccaggctccagggaagaagcgcgagggggtcgcacttattactactgatggtggaaccacactctacgccgactccgtgaagggccgattcaccatctcccaagacaacgccaagaacacggtgtatctgcaaatgaacaacctgaaaccagaggacactgccatgtacacctgtgcggcagacgaccgtccctggtgtatgacggttggtgtgaggacggaagactatgacacctggggccaggggaccctggtcactgtctcatca

SEQ ID NO: 22 - protein, 352 aa, Artificial Sequence
  the amino acid sequence of full-length of 1A5-Fc
QVQLVESGGGSVQAGGSLLLSCAASGYTFSPCAMGWFRQAPGKERSLVSWITVDGTTDYADSVKGRFTISRDNAKNMVYLQMTSLEPEDTATYYCNTVYILTPSCRPQPWGPGTQVTVSSEPKSCDKTHTCPPCPAPELLGGPSVFLFPPKPKDTLMISRTPEVTCVVVDVSHEDPEVKFNWYVDGVEVHNAKTKPREEQYNSTYRVVSVLTVLHQDWLNGKEYKCKVSNKALPAPIEKTISKAKGQPREPQVYTLPPSRDELTKNQVSLTCLVKGFYPSDIAVEWESNGQPENNYKTTPPVLDSDGSFFLYSKLTVDKSRWQQGNVFSCSVMHEALHNHYTQKSLSLSPGK

SEQ ID NO: 23 - DNA, 1056 bp, Artificial Sequence
  the nucleotide sequence of full-length of 1A5-Fc
caagtgcaactggtggagtctggaggcggttccgtgcaggccggcggctccctgctcctgtcctgcgccgcttccggctacaccttctctccttgtgccatgggctggttccggcaggctcctggcaaagaaagatccctggtgtcttggatcaccgtggatggcaccaccgattacgctgactccgtgaagggcagattcaccatctctagagacaacgccaagaacatggtgtacctgcagatgaccagcctggaacctgaggataccgctacctactactgcaacaccgtgtacatcctgacacctagctgccggcctcaaccttggggacctggaacacaggtaaccgtgtcgtccgagcccaagtcttgcgacaagacccacacctgtcctccttgtcctgctccggaactgctgggcggcccttccgtgtttctgtttcctccaaagcctaaggacacactgatgatcagccggacccctgaggtgacctgcgtggtcgtggatgtctctcacgaggatcctgaggtgaagttcaactggtacgtggatggagtggaagtgcataacgctaaaaccaagcctagagaagagcagtacaactccacctacagagtggtgtccgtgctgaccgtgctgcaccaggattggctgaacggcaaagagtacaagtgcaaggtgtccaacaaggctctgcctgcccctatcgagaagaccatctccaaggccaagggccagcctcgggagcctcaagtgtacaccctgcctccttctcgcgacgagctgaccaagaaccaggtgtctctgacctgcctggtgaaaggcttctacccctccgacatcgccgtggaatgggagtccaatggccagcccgagaacaactacaagaccaccccacctgtgctggactctgatggctccttcttcctgtactccaagctgaccgtggacaagtccagatggcagcagggcaacgtgttctcctgttctgtgatgcacgaggccctgcacaaccactacacacagaagtccctgagcctgtctcctggcaag

SEQ ID NO: 24 - protein, 358 aa, Artificial Sequence
  the amino acid sequence of full-length of 1B5-Fc
QVQLVESGGGSVQAGGSLRLSCAASGVTFNSDCMGWFRQAPGKEREAVARIETGYGGTLYADSVKGRFTISRDNAKKTVYLQMNSLKFEDTAMYYCAAKRSWCSPTWWREVDYNYWGQGTLVTVSSEPKSCDKTHTCPPCPAPELLGGPSVFLFPPKPKDTLMISRTPEVTCVVVDVSHEDPEVKFNWYVDGVEVHNAKTKPREEQYNSTYRVVSVLTVLHQDWLNGKEYKCKVSNKALPAPIEKTISKAKGQPREPQVYTLPPSRDELTKNQVSLTCLVKGFYPSDIAVEWESNGQPENNYKTTPPVLDSDGSFFLYSKLTVDKSRWQQGNVFSCSVMHEALHNHYTQKSLSLSPGK

SEQ ID NO: 25 - DNA, 1074 bp, Artificial Sequence
  the nucleotide sequence of full-length of 1B5-Fc
caggtgcagttggttgaatctggcggcggatctgtgcaggctggcggatctctgagactgtcctgtgccgcttccggcgtcaccttcaactccgactgcatgggatggttcagacaggcccctggcaaagagagagaggccgtcgctaggatcgagaccggctatggcggaaccctgtacgccgactccgtcaagggcaggttcaccatcagcagagacaacgccaagaagaccgtgtacctgcagatgaactccctgaagttcgaggacaccgccatgtactactgtgctgccaagagaagctggtgcagccctacctggtggagagaggtggactacaactactggggccagggcacactggtcaccgtgtcctctgagcctaagtcctgcgacaagacccacacctgtcctccatgtcctgctccagaactgctcggcggaccttccgtgttcctgtttcctccaaagcctaaggataccctgatgatctctcggacccctgaagtgacctgcgtggtggtggatgtgtctcacgaggatcccgaagtgaagttcaattggtacgtggacggcgtggaagtgcacaatgctaagaccaagcctagagaggaacagtacaactccacctatagagtggtgtccgtgctgaccgtgctgcaccaggattggctgaacggcaaagagtacaagtgcaaggtgtccaacaaggccctgcctgctcctatcgaaaagaccatctccaaggccaagggccagcctagggaaccccaggtttacaccttgcctccatctcgggacgagctgaccaagaaccaggtgtccctgacctgtctggtcaagggcttctacccctccgatatcgccgtggaatgggagtctaatggccagccagagaacaactacaagacaacccctcctgtgctggactccgacggctcattcttcctgtactccaagctgacagtggacaagtccagatggcagcagggcaacgtgttctcctgctccgtgatgcacgaggccctgcacaatcactacacccagaagtccctgtctctgagccccggcaaa

SEQ ID NO: 26 - protein, 359 aa, Artificial Sequence
  the amino acid sequence of full-length of 1B11-Fc
QVQLVESGGGSVPAGGSMRLSCAASGYRNPMVCMGWFRQAPGKKREGVALITTDGGTTLYADSVKGRFTISQDNAKNTVYLQMNNLKPEDTAMYTCAADDRPWCMTVGVRTEDYDTWGQGTLVTVSSEPKSCDKTHTCPPCPAPELLGGPSVFLFPPKPKDTLMISRTPEVTCVVVDVSHEDPEVKFNWYVDGVEVHNAKTKPREEQYNSTYRVVSVLTVLHQDWLNGKEYKCKVSNKALPAPIEKTISKAKGQPREPQVYTLPPSRDELTKNQVSLTCLVKGFYPSDIAVEWESNGQPENNYKTTPPVLDSDGSFFLYSKLTVDKSRWQQGNVFSCSVMHEALHNHYTQKSLSLSPGK

SEQ ID NO: 27 - DNA, 1077 bp, Artificial Sequence
  the nucleotide sequence of full-length of 1B11-Fc
caggtgcagttggttgaatctggcggcggatctgtgcccgctggcggatctatgagactgtcctgtgccgcttccggctacagaaaccccatggtctgcatgggctggttcagacaggcccctggcaagaagagagaaggcgtcgccctgatcaccaccgatggcggaacaacattgtacgccgactccgtcaagggcaggttcaccatcagccaggacaacgccaagaacaccgtgtacctgcagatgaacaatctgaagcccgaggacaccgccatgtacacctgtgccgccgacgacagaccttggtgtatgaccgtgggcgtcagaaccgaggactacgacacatggggccagggaacactggtcaccgtgtcctctgagcctaagtcctgcgacaagacccacacctgtcctccatgtcctgctccagaactgctcggcggaccttccgtgttcctgtttcctccaaagcctaaggataccctgatgatctctcggacccctgaagtgacctgcgtggtggtggatgtgtctcacgaggatcccgaagtgaagttcaattggtacgtggacggcgtggaagtgcacaatgctaagaccaagcctagagaggaacagtacaactccacctatagagtggtgtccgtgctgaccgtgctgcaccaggattggctgaacggcaaagagtacaagtgcaaggtgtccaacaaggccctgcctgctcctatcgaaaagaccatctccaaggccaagggccagcctagggaaccccaggtttacaccttgcctccatctcgggacgagctgaccaagaaccaggtgtccctgacctgtctggtcaagggcttctacccctccgatatcgccgtggaatgggagtctaatggccagccagagaacaactacaagacaacccctcctgtgctggactccgacggctcattcttcctgtactccaagctgacagtggacaagtccagatggcagcagggcaacgtgttctcctgctccgtgatgcacgaggccctgcacaatcactacacccagaagtccctgtctctgagccccggcaaa